European Patent Application EP 4 198 047 A1, published June 21, 2023. Title: FUKUTIN RELATED PROTEIN GENE TRANSFER INCREASE USING MODIFIED ITR SEQUENCES. Applicant: GENETHON INSTITUT NATIONAL DE LA SANTE ET DE LA RECHERCHE MEDICALE UNIVERSITE D’EVRY VAL D’ESSONNE. The sequence listing filed with the application follows.

SEQUENCE LISTING (12 sequences)

SEQ ID NO: 1 - DNA, 130 bp, Artificial Sequence
  ITRgnt 5'
ctgcgcgctcgctcgctcactgaggccgcccgggcaaagcccgggcgtcgggcgacctttggtcgcccggcctcagtgagcgagcgagcgcgcagagagggagtggccaactccatcactaggggttcct

SEQ ID NO: 2 - DNA, 130 bp, Artificial Sequence
  ITRg 3'
aggaacccctagtgatggagttggccactccctctctgcgcgctcgctcgctcactgaggccgggcgaccaaaggtcgcccgacgcccgggctttgcccgggcggcctcagtgagcgagcgagcgcgcag

SEQ ID NO: 3 - DNA, 1488 bp, Artificial Sequence
  FKRP WT
atgcggctcacccgctgccaggctgccctggcggccgccatcaccctcaaccttctggtcctcttctatgtctcgtggctgcagcaccagcctaggaattcccgggcccgggggccccgtcgtgcctctgctgccggcccccgtgtcaccgtcctggtgcgggagttcgaggcatttgacaacgcggtgcccgagctggtagactccttcctgcagcaagacccagcccagcccgtggtggtggcagccgacacgctcccctacccgcccctggccctgccccgcatccccaacgtgcgtctggcgctgctccagcccgccctggaccggccagccgcagcctcgcgcccggagacctacgtggccaccgagtttgtggccctagtacctgatggggcgcgggctgaggcacctggcctgctggagcgcatggtggaggcgctccgcgcaggaagcgcacgtctggtggccgccccggttgccacggccaaccctgccaggtgcctggccctgaacgtcagcctgcgagagtggaccgcccgctatggcgcagcccccgccgcgccccgctgcgacgccctggacggagatgctgtggtgctcctgcgcgcccgcgacctcttcaacctctcggcgcccctggcccggccggtgggcaccagcctctttctgcagaccgcccttcgcggctgggcggtgcagctgctggacttgaccttcgccgcggcgcgccagcccccgctggccacggcccacgcgcgctggaaggctgagcgcgagggacgcgctcggcgggcggcgctgctccgcgcgctgggcatccgcctagtgagctgggaaggcgggcggctggagtggttcggctgcaacaaggagaccacgcgctgcttcggaaccgtggtgggcgacacgcccgcctacctctacgaggagcgctggacgcccccctgctgcctgcgcgcgctgcgcgagaccgcccgctatgtggtgggcgtgctggaggctgcgggcgtgcgctactggctcgagggcggctcactgctgggggccgcccgccacggggacatcatcccatgggactacgacgtggacctgggcatctacttggaggacgtgggcaactgcgagcagctgcggggggcagaggccggctcggtggtggatgagcgcggcttcgtatgggagaaggcggtcgagggcgactttttccgcgtgcagtacagcgaaagcaaccacttgcacgtggacctgtggcccttctacccccgcaatggcgtcatgaccaaggacacgtggctggaccaccggcaggatgtggagtttcccgagcacttcctgcagccgctggtgcccctgccctttgccggcttcgtggcgcaggcgcctaacaactaccgccgcttcctggagctcaagttcgggcccggggtcatcgagaacccccagtaccccaacccggcactgctgagtctgacgggaagcggctga

SEQ ID NO: 4 - DNA, 1061 bp, Artificial Sequence
  Human Desmin Promoter
taccccctgccccccacagctcctctcctgtgccttgtttcccagccatgcgttctcctctataaatacccgctctggtatttggggttggcagctgttgctgccagggagatggttgggttgacatgcggctcctgacaaaacacaaacccctggtgtgtgtgggcgtgggtggtgtgagtagggggatgaatcagggagggggcgggggacccagggggcaggagccacacaaagtctgtgcgggggtgggagcgcacatagcaattggaaactgaaagcttatcagaccctttctggaaatcagcccactgtttataaacttgaggccccaccctcgacagtaccggggaggaagagggcctgcactagtccagagggaaactgaggctcagggctagctcgcccatagacatacatggcaggcaggctttggccaggatccctccgcctgccaggcgtctccctgccctcccttcctgcctagagacccccaccctcaagcctggctggtctttgcctgagacccaaacctcttcgacttcaagagaatatttaggaacaaggtggtttagggcctttcctgggaacaggccttgaccctttaagaaatgacccaaagtctctccttgaccaaaaaggggaccctcaaactaaagggaagcctctcttctgctgtctcccctgaccccactcccccccaccccaggacgaggagataaccagggctgaaagaggcccgcctgggggctgcagacatgcttgctgcctgccctggcgaaggattggcaggcttgcccgtcacaggacccccgctggctgactcaggggcgcaggcctcttgcgggggagctggcctccccgcccccacggccacgggccgccctttcctggcaggacagcgggatcttgcagctgtcaggggaggggaggcgggggctgatgtcaggagggatacaaatagtgccgacggctgggggccctgtctcccctcgccgcatccactctccggccggccgcctgcccgccgcctcctccgtgcgcccgccagcctcgcccgc

SEQ ID NO: 5 - DNA, 762 bp, Artificial Sequence
  pA-HBB2
accccaccagtgcaggctgcctatcagaaagtggtggctggtgtggctaatgccctggcccacaagtatcactaagctcgctttcttgctgtccaatttctattaaaggttcctttgttccctaagtccaactactaaactgggggatattatgaagggccttgagcatctggattctgcctaataaaaaacatttattttcattgcaatgatgtatttaaattatttctgaatattttactaaaaagggaatgtgggaggtcagtgcatttaaaacataaagaaatgaagagctagttcaaaccttgggaaaatacactatatcttaaactccatgaaagaaggtgaggctgcaaacagctaatgcacattggcaacagccctgatgcctatgccttattcatccctcagaaaaggattcaagtagaggcttgatttggaggttaaagttttgctatgctgtattttacattacttattgttttagctgtcctcatgaatgtcttttcactacccatttgcttatcctgcatctctcagccttgactccactcagttctcttgcttagagataccacctttcccctgaagtgttccttccatgttttacggcgagatggtttctcctcgcctggccactcagccttagttgtctctgttgtcttatagaggtctacttgaagaaggaaaaacagggggcatggtttgactgtcctgtgagcccttcttccctgcctcccccactcacagtgacccggaatc

SEQ ID NO: 6 - DNA, 1488 bp, Artificial Sequence
  FKRP-opt2-mini
atgcggctcacccgctgccaggctgccctggcggccgccatcaccctcaaccttctggtcctcttctatgtctcgtggctgcagcaccagcctaggaattcccgggcccgggggccccgtcgtgcctctgctgccggcccccgtgtcaccgtcctggtgcgggagttcgaggcatttgacaacgcggtgcccgagctggtagactccttcctgcagcaagacccagcccagcccgtggtggtggcagccgacacgctcccctacccgcccctggccctgccccgcatccccaacgtgcgtctggcgctgctccagcccgccctggaccggccagccgcagcctcgcgcccggagacctacgtggccaccgagtttgtggccctagtacctgatggggcgcgggctgaggcacctggcctgctggagcggatggtggaggcgctccgcgcaggaagcgcacgtctggtggccgccccggttgccacggccaaccctgccaggtgcctggccctgaacgtcagcctgcgagagtggaccgcccgctacggcgcagcccccgccgcgccccgctgcgacgccctggacggagatgctgtggtgctcctgcgcgcccgcgacctcttcaacctctcggcgcccctggcccggccggtgggcaccagcctctttctgcagaccgcccttcgcggctgggcggtgcagctgctggacttgaccttcgccgcggcgcgccagcccccgctggccacggcccacgcgcgctggaaggctgagcgcgagggacgcgctcggcgggcggcgctgctccgcgcgctgggaatccgcctagtgagctgggaaggcgggcggctggagtggttcggctgcaacaaggagaccacgcgctgcttcggaaccgtggtgggcgacacgcccgcctacctctacgaggagcgctggacgcccccctgctgcctgcgcgcgctgcgcgagaccgcccgctatgtggtgggcgtgctggaggctgcgggcgtgcgctactggctcgagggcggctcactgctgggggccgcccgccacggggacatcatcccatgggactacgacgtggacctgggcatctacttggaggacgtgggcaactgcgagcagctgcggggggcagaggccggctcggtggtggatgagcgcggcttcgtatgggagaaggcggtcgagggcgactttttccgcgtgcagtacagcgaaagcaaccacttgcacgtggacctgtggcccttctacccccgcaatggcgtcatgaccaaggacacgtggctggaccaccggcaggatgtggagtttcccgagcacttcctgcagccgctggtgcccctgccctttgccggcttcgtggcgcaggcgcctaacaactaccgccgcttcctggagctcaagttcgggcccggggtgatcgagaacccccagtaccccaacccggcactgctgagtctgacgggaagcggctga

SEQ ID NO: 7 - DNA, 1488 bp, Artificial Sequence
  FKRP-opt2-comp
atgagactgaccaggtgccaggctgccctggctgctgccatcaccctgaacctgctggtgctgttctatgtgagctggctgcagcaccagcccaggaacagcagggccaggggccccaggagggcctctgctgctggccccagggtgacagtgctggtgagggagtttgaggcctttgacaatgctgtgcctgagctggtggacagcttcctgcagcaggaccctgcccagcctgtggtggtggctgctgataccctgccctacccccccctggccctgcccaggatccccaatgtgaggctggccctgctgcagcctgccctggacaggcctgctgctgccagcaggcctgagacctatgtggccacagagtttgtggccctggtgcctgatggggccagggctgaggcccctggcctgctggagaggatggtggaggccctgagggctggctctgccaggctggtggctgcccctgtggccacagccaaccctgccaggtgcctggccctgaatgtgagcctgagagagtggacagccaggtatggggctgcccctgctgcccccaggtgtgatgccctggatggagatgctgtggtgctgctgagggccagggacctgttcaacctgtctgcccccctggccaggcctgtggggaccagcctgtttctgcagacagccctgaggggctgggctgtgcagctgctggacctgacctttgctgctgccaggcagccccccctggctacagcccacgccaggtggaaggctgagagggagggcagggccaggagggctgccctgctgagggccctggggatcaggctggtgagctgggaggggggcaggctggagtggtttggctgcaacaaggagacaaccaggtgctttgggacagtggtgggggatacccctgcctacctgtatgaggagaggtggacccccccctgctgcctgagggccctgagggagacagccaggtatgtggtgggggtgctggaggctgctggggtgaggtactggctggaggggggcagcctgctgggggctgccaggcacggggacattatcccctgggactatgatgtggacctgggcatctacctggaggatgtgggcaactgtgagcagctgaggggggctgaggctggctctgtggtggatgagaggggctttgtgtgggagaaggctgtggagggggactttttcagggtgcagtactctgagagcaaccacctgcacgtggacctgtggcccttctaccccaggaatggggtgatgaccaaggacacctggctggaccacaggcaggatgtggagttccctgagcacttcctgcagcccctggtgcccctgccctttgctggctttgtggcccaggcccccaacaactacaggaggttcctggagctgaagtttggccctggggtgattgagaacccccagtaccccaaccctgccctgctgagcctgacaggctctggctga

SEQ ID NO: 8 - DNA, 1488 bp, Artificial Sequence
  FKRP-06
atgagactgacaagatgccaggccgccctggccgctgccatcacactgaatctgctggtgctgttctatgtgtcctggctgcagcaccagccccggaactctagagccagaggcccaagaagggcctctgccgccggacctagagtgacagtgctcgtgcgcgagttcgaggccttcgacaatgccgtgcccgagctggtggacagcttcctgcagcaagaccctgctcagcctgtggtggtggccgccgatacactgccttatcctccactggccctgcccagaatccccaatgtgcgactggctctgctgcagcccgccctggatagacctgccgccgctagcagacctgagacatacgtggccaccgagttcgtggccctggtgcctgatggcgccagagctgaagctcccggcctgctggaaagaatggtggaagccctgagagccggcagcgccagactggtggctgctcctgtggctaccgccaaccctgccagatgtctggccctgaatgtgtccctgagagagtggaccgccagatacggcgctgcccctgccgctcctagatgtgatgctctggatggcgacgccgtggtgctgctgagagccagggacctgttcaacctgagcgcccctctggccagacctgtgggcacaagcctgtttctgcagacagccctgaggggctgggccgtgcagctgctggatctgacatttgccgctgccagacagcctcctctggccacagcccatgccagatggaaggccgagagagagggcagagccagaagggctgctctgctgagggccctgggcatcagactggtgtcttgggaaggcggcagactcgagtggttcggctgcaacaaagaaaccacccggtgcttcggcaccgtcgtgggcgatacaccagcctacctgtacgaggaaagatggacccccccttgctgcctgcgggccctgagagaaacagccagatatgtcgtgggcgtgctggaagccgctggcgtgcgatattggctggaaggcggatctctgctgggagccgccaggcacggcgacatcatcccttgggactacgacgtggacctgggcatctacctggaagatgtgggcaactgcgagcagctgagaggcgccgaagccggctctgtggtggatgagaggggcttcgtgtgggagaaggccgtggaaggcgacttcttccgggtgcagtacagcgagagcaaccatctgcatgtggacctgtggcccttctacccccggaacggcgtgatgaccaaggacacctggctggaccaccggcaggacgtggaattccccgagcactttctgcagcccctggtgccactgcctttcgccggatttgtggcccaggcccccaacaactaccggcggttcctggaactgaagttcggccctggcgtgatcgagaacccccagtaccctaaccctgccctgctgagcctgaccggcagcggctaa

SEQ ID NO: 9 - DNA, 1488 bp, Artificial Sequence
  FKRP-07
atgcggctcacccgctgccaggctgccctggctgccgccatcaccctcaaccttctggtcctcttctatgtcagctggctgcagcaccagcctaggaattcccgggcccgggggcccaggagggcctctgctgccggccccagggtcaccgtcctggtgcgggagttcgaggcatttgacaacgctgtgcccgagctggtagactccttcctgcagcaagacccagcccagcccgtggtggtggcagccgacaccctcccctacccccccctggccctgccccgcatccccaacgtgaggctggccctgctccagcccgccctggaccggccagccgcagccagccgccctgagacctacgtggccaccgagtttgtggccctggtacctgatggggcccgggctgaggcacctggcctgctggagcggatggtggaggccctccgcgcaggaagcgcaaggctggtggccgcccctgttgccacagccaaccctgccaggtgcctggccctgaacgtcagcctgcgagagtggaccgcccgctacggcgcagcccccgccgccccccgctgcgacgccctggacggagatgctgtggtgctcctgcgcgcccgcgacctcttcaacctctctgcccccctggcccggcctgtgggcaccagcctctttctgcagaccgcccttcgcggctgggctgtgcagctgctggacttgaccttcgccgctgcccgccagccccccctggccacagcccacgcccgctggaaggctgagcgcgagggacgcgctcggcgggctgccctgctccgcgccctgggaatccgcctggtgagctgggaaggcgggcggctggagtggttcggctgcaacaaggagaccacccgctgcttcggaaccgtggtgggcgacacccccgcctacctctacgaggagcgctggacccccccctgctgcctgcgcgccctgcgcgagaccgcccgctatgtggtgggcgtgctggaggctgctggcgtgcgctactggctcgagggcggctcactgctgggggccgcccgccacggggacatcatcccatgggactacgacgtggacctgggcatctacttggaggacgtgggcaactgcgagcagctgcggggggcagaggccggctctgtggtggatgagcgcggcttcgtatgggagaaggctgtcgagggcgactttttccgcgtgcagtacagcgaaagcaaccacttgcacgtggacctgtggcccttctacccccgcaatggcgtcatgaccaaggacacctggctggaccaccggcaggatgtggagtttcccgagcacttcctgcagcccctggtgcccctgccctttgccggcttcgtggcccaggcccctaacaactaccgccgcttcctggagctcaagttcgggcccggggtgatcgagaacccccagtaccccaaccctgcactgctgagtctgaccggaagcggctga

SEQ ID NO: 10 - DNA, 1488 bp, Artificial Sequence
  FKRP-08
atgcggctcacccgctgccaggctgccctggctgctgccatcaccctcaaccttctggtcctcttctatgtcagctggctgcagcaccagcctaggaattcccgggcccgggggcccaggagggcctctgctgctggccccagggtcaccgtcctggtgcgggagttcgaggcatttgacaacgctgtgcccgagctggtagactccttcctgcagcaagacccagcccagcccgtggtggtggcagctgacaccctcccctacccccccctggccctgccccgcatccccaacgtgaggctggccctgctccagcccgccctggaccggccagctgcagccagccgccctgagacctacgtggccaccgagtttgtggccctggtacctgatggggcccgggctgaggcacctggcctgctggagcggatggtggaggccctcagggcaggaagcgcaaggctggtggctgcccctgttgccacagccaaccctgccaggtgcctggccctgaacgtcagcctgcgagagtggaccgcccgctacggggcagcccccgctgccccccgctgcgacgccctggacggagatgctgtggtgctcctgagggccagggacctcttcaacctctctgcccccctggcccggcctgtgggcaccagcctctttctgcagaccgcccttaggggctgggctgtgcagctgctggacttgaccttcgctgctgcccgccagccccccctggccacagcccacgcccgctggaaggctgagagggagggaagggctcggcgggctgccctgctcagggccctgggaatccgcctggtgagctgggaaggggggcggctggagtggttcggctgcaacaaggagaccacccgctgcttcggaaccgtggtgggggacacccccgcctacctctacgaggagcgctggacccccccctgctgcctgagggccctgagggagaccgcccgctatgtggtgggggtgctggaggctgctggggtgcgctactggctcgaggggggctcactgctgggggctgcccgccacggggacatcatcccatgggactacgacgtggacctgggcatctacttggaggacgtgggcaactgcgagcagctgcggggggcagaggctggctctgtggtggatgagaggggcttcgtatgggagaaggctgtggagggggactttttcagggtgcagtacagcgaaagcaaccacttgcacgtggacctgtggcccttctacccccgcaatggggtcatgaccaaggacacctggctggaccaccggcaggatgtggagtttcccgagcacttcctgcagcccctggtgcccctgccctttgctggcttcgtggcccaggcccctaacaactaccgccgcttcctggagctcaagttcgggcccggggtgatcgagaacccccagtaccccaaccctgcactgctgagtctgaccggaagcggctga

SEQ ID NO: 11 - DNA, 1488 bp, Artificial Sequence
  FKRP-10
atgagactgacaaggtgccaggctgccctggctgctgccatcacactgaacctgctggtgctgttttatgtgagctggctgcagcaccagcctaggaacagcagggccaggggccctaggagggcctctgctgctggccctagggtgacagtgctggtgagggagtttgaggcctttgacaatgctgtgcctgagctggtggacagctttctgcagcaggaccctgcccagcctgtggtggtggctgctgatacactgccttaccctcctctggccctgcctaggatccctaatgtgaggctggccctgctgcagcctgccctggacaggcctgctgctgccagcaggcctgagacttatgtggccacagagtttgtggccctggtgcctgatggggccagggctgaggcccctggcctgctggagaggatggtggaggccctgagggctggctctgccaggctggtggctgcccctgtggccacagccaaccctgccaggtgcctggccctgaatgtgagcctgagagagtggacagccaggtatggggctgcccctgctgcccctaggtgtgatgccctggatggagatgctgtggtgctgctgagggccagggacctgtttaacctgtctgcccctctggccaggcctgtggggacaagcctgtttctgcagacagccctgaggggctgggctgtgcagctgctggacctgacatttgctgctgccaggcagcctcctctggctacagcccacgccaggtggaaggctgagagggagggcagggccaggagggctgccctgctgagggccctggggatcaggctggtgagctgggaggggggcaggctggagtggtttggctgcaacaaggagacaacaaggtgctttgggacagtggtgggggatacacctgcctacctgtatgaggagaggtggacacctccttgctgcctgagggccctgagggagacagccaggtatgtggtgggggtgctggaggctgctggggtgaggtactggctggaggggggcagcctgctgggggctgccaggcacggggacattatcccttgggactatgatgtggacctgggcatctacctggaggatgtgggcaactgtgagcagctgaggggggctgaggctggctctgtggtggatgagaggggctttgtgtgggagaaggctgtggagggggacttttttagggtgcagtactctgagagcaaccacctgcacgtggacctgtggcctttttaccctaggaatggggtgatgacaaaggacacatggctggaccacaggcaggatgtggagtttcctgagcactttctgcagcctctggtgcctctgccttttgctggctttgtggcccaggcccctaacaactacaggaggtttctggagctgaagtttggccctggggtgattgagaaccctcagtaccctaaccctgccctgctgagcctgacaggctctggctga

SEQ ID NO: 12 - DNA, 1488 bp, Artificial Sequence
  FKRP-11
atgagactgacaaggtgccaggctgccctggctgctgccatcacactgaacctgctggtgctgttttatgtgagctggctgcagcaccagcctagaaacagcagagccagaggccctagaagagcctctgctgctggccctagagtgacagtgctggtgagagagtttgaggcctttgacaatgctgtgcctgagctggtggacagctttctgcagcaggaccctgcccagcctgtggtggtggctgctgatacactgccttaccctcctctggccctgcctagaatccctaatgtgagactggccctgctgcagcctgccctggacagacctgctgctgccagcagacctgagacttatgtggccacagagtttgtggccctggtgcctgatggggccagagctgaggcccctggcctgctggagagaatggtggaggccctgagagctggctctgccagactggtggctgcccctgtggccacagccaaccctgccagatgcctggccctgaatgtgagcctgagagagtggacagccagatatggggctgcccctgctgcccctagatgtgatgccctggatggagatgctgtggtgctgctgagagccagagacctgtttaacctgtctgcccctctggccagacctgtggggacaagcctgtttctgcagacagccctgagaggctgggctgtgcagctgctggacctgacatttgctgctgccagacagcctcctctggctacagcccacgccagatggaaggctgagagagagggcagagccagaagagctgccctgctgagagccctggggatcaggctggtgagctgggaggggggcagactggagtggtttggctgcaacaaggagacaacaagatgctttgggacagtggtgggggatacacctgcctacctgtatgaggagaggtggacacctccttgctgcctgagagccctgagagagacagccagatatgtggtgggggtgctggaggctgctggggtgagatactggctggaggggggcagcctgctgggggctgccagacacggggacattatcccttgggactatgatgtggacctgggcatctacctggaggatgtgggcaactgtgagcagctgagaggggctgaggctggctctgtggtggatgagagaggctttgtgtgggagaaggctgtggagggggacttttttagagtgcagtactctgagagcaaccacctgcacgtggacctgtggcctttttaccctagaaatggggtgatgacaaaggacacatggctggaccacagacaggatgtggagtttcctgagcactttctgcagcctctggtgcctctgccttttgctggctttgtggcccaggcccctaacaactacagaagatttctggagctgaagtttggccctggggtgattgagaaccctcagtaccctaaccctgccctgctgagcctgacaggctctggctga